European Patent Specification EP 4 267 245 B1, published February 26, 2025. Title: Method. Applicant: Agency for Science, Technology and Research Tan Tock Seng Hospital Pte Ltd BARD, Frederic TRAN, Le Son LEONG, Khai Pang. The sequence listing filed with the application follows.

SEQUENCE LISTING (11 sequences)

SEQ ID NO: 1 - DNA, 9522 bp, Artificial Sequence
  ER-2Lec
aatgtagtcttatgcaatactcttgtagtcttgcaacatggtaacgatgagttagcaacatgccttacaaggagagaaaaagcaccgtgcatgccgattggtggaagtaaggtggtacgatcgtgccttattaggaaggcaacagacgggtctgacatggattggacgaaccactgaattgccgcattgcagagatattgtatttaagtgcctagctcgatacataaacgggtctctctggttagaccagatctgagcctgggagctctctggctaactagggaacccactgcttaagcctcaataaagcttgccttgagtgcttcaagtagtgtgtgcccgtctgttgtgtgactctggtaactagagatccctcagacccttttagtcagtgtggaaaatctctagcagtggcgcccgaacagggacttgaaagcgaaagggaaaccagaggagctctctcgacgcaggactcggcttgctgaagcgcgcacggcaagaggcgaggggcggcgactggtgagtacgccaaaaattttgactagcggaggctagaaggagagagatgggtgcgagagcgtcagtattaagcgggggagaattagatcgcgatgggaaaaaattcggttaaggccagggggaaagaaaaaatataaattaaaacatatagtatgggcaagcagggagctagaacgattcgcagttaatcctggcctgttagaaacatcagaaggctgtagacaaatactgggacagctacaaccatcccttcagacaggatcagaagaacttagatcattatataatacagtagcaaccctctattgtgtgcatcaaaggatagagataaaagacaccaaggaagctttagacaagatagaggaagagcaaaacaaaagtaagaccaccgcacagcaagcggccgctgatcttcagacctggaggaggagatatgagggacaattggagaagtgaattatataaatataaagtagtaaaaattgaaccattaggagtagcacccaccaaggcaaagagaagagtggtgcagagagaaaaaagagcagtgggaataggagctttgttccttgggttcttgggagcagcaggaagcactatgggcgcagcgtcaatgacgctgacggtacaggccagacaattattgtctggtatagtgcagcagcagaacaatttgctgagggctattgaggcgcaacagcatctgttgcaactcacagtctggggcatcaagcagctccaggcaagaatcctggctgtggaaagatacctaaaggatcaacagctcctggggatttggggttgctctggaaaactcatttgcaccactgctgtgccttggaatgctagttggagtaataaatctctggaacagatttggaatcacacgacctggatggagtgggacagagaaattaacaattacacaagcttaatacactccttaattgaagaatcgcaaaaccagcaagaaaagaatgaacaagaattattggaattagataaatgggcaagtttgtggaattggtttaacataacaaattggctgtggtatataaaattattcataatgatagtaggaggcttggtaggtttaagaatagtttttgctgtactttctatagtgaatagagttaggcagggatattcaccattatcgtttcagacccacctcccaaccccgaggggacccgacaggcccgaaggaatagaagaagaaggtggagagagagacagagacagatccattcgattagtgaacggatctcgacggtatcggttaacttttaaaagaaaaggggggattggggggtacagtgcaggggaaagaatagtagacataatagcaacagacatacaaactaaagaattacaaaaacaaattacaaaaattcaaaattttatcgataagcttgggagttccgcgttacataacttacggtaaatggcccgcctggctgaccgcccaacgacccccgcccattgacgtcaataatgacgtatgttcccatagtaacgccaatagggactttccattgacgtcaatgggtggagtatttacggtaaactgcccacttggcagtacatcaagtgtatcatatgccaagtacgccccctattgacgtcaatgacggtaaatggcccgcctggcattatgcccagtacatgaccttatgggactttcctacttggcagtacatctacgtattagtcatcgctattaccatggtgatgcggttttggcagtacatcaatgggcgtggatagcggtttgactcacggggatttccaagtctccaccccattgacgtcaatgggagtttgttttggcaccaaaatcaacgggactttccaaaatgtcgtaacaactccgccccattgacgcaaatgggcggtaggcgtgtacggtgggaggtctatataagcagagctcgtttagtgaaccgtcagatcgcctggagacgccatccacgctgttttgacctccatagaagacaccgggaccgatccagcctccggactctagaggatccctaccggtgatatcctcgagaccatggctacaggctcccggacgtccctgctcctggcttttggcctgctctgcctgccctggcttcaagagggcagtgccttcccaaccattcccttatccgtgagcaagggcgaggagctgttcaccggggtggtgcccatcctggtcgagctggacggcgacgtaaacggccacaagttcagcgtgtccggcgagggcgagggcgatgccacctacggcaagctgaccctgaagttcatctgcaccaccggcaagctgcccgtgccctggcccaccctcgtgaccaccttcacctacggcgtgcagtgcttcgcccgctaccccgaccacatgaagcagcacgacttcttcaagtccgccatgcccgaaggctacgtccaggagcgcaccatcttcttcaaggacgacggcaactacaagacccgcgccgaggtgaagttcgagggcgacaccctggtgaaccgcatcgagctgaagggcatcgacttcaaggaggacggcaacatcctggggcacaagctggagtacaactacaacagccacaaggtctatatcaccgccgacaagcagaagaacggcatcaaggtgaacttcaagacccgccacaacatcgaggacggcagcgtgcagctcgccgaccactaccagcagaacacccccatcggcgacggccccgtgctgctgcccgacaaccactacctgagcacccagtccgccctgagcaaagaccccaacgagaagcgcgatcacatggtcctgctggagttcgtgaccgccgccgggatcactctcggcatggacgagctgtacaagggctcgagcccatcaacaagtttgtacaaaaaagcaggctccgataacgggaagcctatccctaaccctctcctcggtctcgattctacggagttaagggttccagaccatcaggatatagcttttggggccttgcagcagggaactaactgcctcgacactttgggacactttgctgatggtgtggttggagtttatgaatgtcacaatgctgggggaaaccaggaatgggccttgacgaaggagaagtcggtgaagcacatggatttgtgccttactgtggtggaccgggcaccgggctctcttataaagctgcagggctgccgagaaaatgacagcagacagaaatgggaacagatcgagggcaactccaagctgaggcacgtgggcagcaacctgtgcctggacagtcgcacggccaagagcgggggcctaagcgtggaggtgtgtggcccggccctttcgcagcagtggaagttcacgctcaacctgcagcaggcacagggagcccaagggagatccgataacgggaagcctatccctaaccctctcctcggtctcgattctacggagttaagggttccagaccatcaggatatagcttttggggccttgcagcagggaactaactgcctcgacactttgggacactttgctgatggtgtggttggagtttatgaatgtcacaatgctgggggaaaccaggaatgggccttgacgaaggagaagtcggtgaagcacatggatttgtgccttactgtggtggaccgggcaccgggctctcttataaagctgcagggctgccgagaaaatgacagcagacagaaatgggaacagatcgagggcaactccaagctgaggcacgtgggcagcaacctgtgcctggacagtcgcacggccaagagcgggggcctaagcgtggaggtgtgtggcccggccctttcgcagcagtggaagttcacgctcaacctgcagcagaaagacgagctgtaggacccagctttcttgtacaaagtggttgatatccagcacagtggcggccgctcgagtctagagggcccgcggttcgaaggtaagcctatccctaaccctctcctcggtctcgattctacgcgtaccggttagtaatgatcgacaatcaacctctggattacaaaatttgtgaaagattgactggtattcttaactatgttgctccttttacgctatgtggatacgctgctttaatgcctttgtatcatgctattgcttcccgtatggctttcattttctcctccttgtataaatcctggttgctgtctctttatgaggagttgtggcccgttgtcaggcaacgtggcgtggtgtgcactgtgtttgctgacgcaacccccactggttggggcattgccaccacctgtcagctcctttccgggactttcgctttccccctccctattgccacggcggaactcatcgccgcctgccttgcccgctgctggacaggggctcggctgttgggcactgacaattccgtggtgttgtcggggaagctgacgtcctttccatggctgctcgcctgtgttgccacctggattctgcgcgggacgtccttctgctacgtcccttcggccctcaatccagcggaccttccttcccgcggcctgctgccggctctgcggcctcttccgcgtcttcgccttcgccctcagacgagtcggatctccctttgggccgcctccccgcctggcgatggtaccggtgtggaaagtccccaggctccccagcaggcagaagtatgcaaagcatgcatctcaattagtcagcaaccaggtgtggaaagtccccaggctccccagcaggcagaagtatgcaaagcatgcatctcaattagtcagcaaccatagtcccgcccctaactccgcccatcccgcccctaactccgcccagttccgcccattctccgccccatggctgactaattttttttatttatgcagaggccgaggccgcctctgcctctgagctattccagaagtagtgaggaggcttttttggaggcctaggcttttgcaaaaagctcccgggagcttgtatatccattttcggatctgatcagcacgtgttgacaattaatcatcggcatagtatatcggcatagtataatacgacaaggtgaggaactaaaccatggccaagcctttgtctcaagaagaatccaccctcattgaaagagcaacggctacaatcaacagcatccccatctctgaagactacagcgtcgccagcgcagctctctctagcgacggccgcatcttcactggtgtcaatgtatatcattttactgggggaccttgtgcagaactcgtggtgctgggcactgctgctgctgcggcagctggcaacctgacttgtatcgtcgcgatcggaaatgagaacaggggcatcttgagcccctgcggacggtgccgacaggtgcttctcgatctgcatcctgggatcaaagccatagtgaaggacagtgatggacagccgacggcagttgggattcgtgaattgctgccctctggttatgtgtgggagggctaagcacaattcgagctcggtacctttaagaccaatgacttacaaggcagctgtagatcttagccactttttaaaagaaaaggggggactggaagggctaattcactcccaacgaagacaagatctgctttttgcttgtactgggtctctctggttagaccagatctgagcctgggagctctctggctaactagggaacccactgcttaagcctcaataaagcttgccttgagtgcttcaagtagtgtgtgcccgtctgttgtgtgactctggtaactagagatccctcagacccttttagtcagtgtggaaaatctctagcagtagtagttcatgtcatcttattattcagtatttataacttgcaaagaaatgaatatcagagagtgagaggaacttgtttattgcagcttataatggttacaaataaagcaatagcatcacaaatttcacaaataaagcatttttttcactgcattctagttgtggtttgtccaaactcatcaatgtatcttatcatgtctggctctagctatcccgcccctaactccgcccatcccgcccctaactccgcccagttccgcccattctccgccccatggctgactaattttttttatttatgcagaggccgaggccgcctcggcctctgagctattccagaagtagtgaggaggcttttttggaggcctagggacgtacccaattcgccctatagtgagtcgtattacgcgcgctcactggccgtcgttttacaacgtcgtgactgggaaaaccctggcgttacccaacttaatcgccttgcagcacatccccctttcgccagctggcgtaatagcgaagaggcccgcaccgatcgcccttcccaacagttgcgcagcctgaatggcgaatgggacgcgccctgtagcggcgcattaagcgcggcgggtgtggtggttacgcgcagcgtgaccgctacacttgccagcgccctagcgcccgctcctttcgctttcttcccttcctttctcgccacgttcgccggctttccccgtcaagctctaaatcgggggctccctttagggttccgatttagtgctttacggcacctcgaccccaaaaaacttgattagggtgatggttcacgtagtgggccatcgccctgatagacggtttttcgccctttgacgttggagtccacgttctttaatagtggactcttgttccaaactggaacaacactcaaccctatctcggtctattcttttgatttataagggattttgccgatttcggcctattggttaaaaaatgagctgatttaacaaaaatttaacgcgaattttaacaaaatattaacgcttacaatttaggtggcacttttcggggaaatgtgcgcggaacccctatttgtttatttttctaaatacattcaaatatgtatccgctcatgagacaataaccctgataaatgcttcaataatattgaaaaaggaagagtatgagtattcaacatttccgtgtcgcccttattcccttttttgcggcattttgccttcctgtttttgctcacccagaaacgctggtgaaagtaaaagatgctgaagatcagttgggtgcacgagtgggttacatcgaactggatctcaacagcggtaagatccttgagagttttcgccccgaagaacgttttccaatgatgagcacttttaaagttctgctatgtggcgcggtattatcccgtattgacgccgggcaagagcaactcggtcgccgcatacactattctcagaatgacttggttgagtactcaccagtcacagaaaagcatcttacggatggcatgacagtaagagaattatgcagtgctgccataaccatgagtgataacactgcggccaacttacttctgacaacgatcggaggaccgaaggagctaaccgcttttttgcacaacatgggggatcatgtaactcgccttgatcgttgggaaccggagctgaatgaagccataccaaacgacgagcgtgacaccacgatgcctgtagcaatggcaacaacgttgcgcaaactattaactggcgaactacttactctagcttcccggcaacaattaatagactggatggaggcggataaagttgcaggaccacttctgcgctcggcccttccggctggctggtttattgctgataaatctggagccggtgagcgtgggtctcgcggtatcattgcagcactggggccagatggtaagccctcccgtatcgtagttatctacacgacggggagtcaggcaactatggatgaacgaaatagacagatcgctgagataggtgcctcactgattaagcattggtaactgtcagaccaagtttactcatatatactttagattgatttaaaacttcatttttaatttaaaaggatctaggtgaagatcctttttgataatctcatgaccaaaatcccttaacgtgagttttcgttccactgagcgtcagaccccgtagaaaagatcaaaggatcttcttgagatcctttttttctgcgcgtaatctgctgcttgcaaacaaaaaaaccaccgctaccagcggtggtttgtttgccggatcaagagctaccaactctttttccgaaggtaactggcttcagcagagcgcagataccaaatactgttcttctagtgtagccgtagttaggccaccacttcaagaactctgtagcaccgcctacatacctcgctctgctaatcctgttaccagtggctgctgccagtggcgataagtcgtgtcttaccgggttggactcaagacgatagttaccggataaggcgcagcggtcgggctgaacggggggttcgtgcacacagcccagcttggagcgaacgacctacaccgaactgagatacctacagcgtgagctatgagaaagcgccacgcttcccgaagggagaaaggcggacaggtatccggtaagcggcagggtcggaacaggagagcgcacgagggagcttccagggggaaacgcctggtatctttatagtcctgtcgggtttcgccacctctgacttgagcgtcgatttttgtgatgctcgtcaggggggcggagcctatggaaaaacgccagcaacgcggcctttttacggttcctggccttttgctggccttttgctcacatgttctttcctgcgttatcccctgattctgtggataaccgtattaccgcctttgagtgagctgataccgctcgccgcagccgaacgaccgagcgcagcgagtcagtgagcgaggaagcggaagagcgcccaatacgcaaaccgcctctccccgcgcgttggccgattcattaatgcagctggcacgacaggtttcccgactggaaagcgggcagtgagcgcaacgcaattaatgtgagttagctcactcattaggcaccccaggctttacactttatgcttccggctcgtatgttgtgtggaattgtgagcggataacaatttcacacaggaaacagctatgaccatgattacgccaagcgcgcaattaaccctcactaaagggaacaaaagctggagctgcaagctt

SEQ ID NO: 2 - RNA, 21 nt, Artificial Sequence
  siRNA target sequence for Calnexin (CNX)
caagagugguccuaggagauu

SEQ ID NO: 3 - RNA, 19 nt, Artificial Sequence
  siRNA target sequence for PDIA3
ggaauagucccauuagcaa

SEQ ID NO: 4 - RNA, 19 nt, Artificial Sequence
  siRNA target sequence for PDIA3
gggcaaggacuuacuuauu

SEQ ID NO: 5 - RNA, 19 nt, Artificial Sequence
  siRNA target sequence for PDIA3
agacccaaauaucgucaua

SEQ ID NO: 6 - RNA, 18 nt, Artificial Sequence
  siRNA target sequence for PDIA3
aggaguucucgcgugaug

SEQ ID NO: 7 - RNA, 19 nt, Artificial Sequence
  siRNA target sequence for PDIA3
gaacgaguaugaugauaau

SEQ ID NO: 8 - RNA, 19 nt, Artificial Sequence
  siRNA target sequence for PDIA3
ggacaagacuguggcauau

SEQ ID NO: 9 - RNA, 19 nt, Artificial Sequence
  siRNA target sequence for PDIA3
ggcaaggacuuacuuauug

SEQ ID NO: 10 - RNA, 19 nt, Artificial Sequence
  siRNA target sequence for PDIA3
ugauaaagaugccucuaua

SEQ ID NO: 11 - protein, 16 aa, Artificial Sequence
  (DOX) inducible 2 lectin domains of GALNT2
TPTTVGPTTVGSTTVG